European Patent Application EP 4 417 621 A1, published August 21, 2024. Title: DESIGN AND APPLICATION OF FULLY HUMAN ANTIBODY FOR NEUTRALIZING RESPIRATORY SYNCYTIAL VIRUS. Applicant: CENTER FOR EXCELLENCE IN MOLECULAR CELL SCIENCE, CHINESE ACADEMY OF SCIENCES. The sequence listing filed with the application follows.

SEQUENCE LISTING (20 sequences)

SEQ ID NO: 1 - protein, 126 aa, synthetic construct
  source 1..126: note = Heavy chain variable region of 4F1 germline reversion
QVQLVESGGGVVQPGRSLRLSCAASGFSFYSYSVHWVRQAPGKGLEWVADVVYDGNHQHYTDSVKGRFTISRDTSKNTVYLQMGSLRAEDTALYYCTARSLVITLAGAGRDDYWGQGTTVTVSSAS

SEQ ID NO: 2 - protein, 126 aa, synthetic construct
  source 1..126: note = Heavy chain variable region of 4F1En1
QVQLVESGGGVVQPGRSLRLSCAASGFSFYSYSVHWVRQAPGKGLEWVADVVYDGNHQHYTDSVKGRFTISRDTRKNTVYLQMGSLRAEDTALYYCTARSLVITLAGAGRDDYWGQGTTVTVSSAS

SEQ ID NO: 3 - protein, 126 aa, synthetic construct
  source 1..126: note = Heavy chain variable region of 4F1En2
QVQLVESGGGVVQPGRSLRLSCAASGFSFYSYSVHWVRQAPGKGLEWVADVVYDGNHQHYTDSVKGRFTISRDTRKNTVYLQMGSLRAEDTALYYCTARSLSITLAGAGRDDYWGQGTTVTVSSAS

SEQ ID NO: 4 - protein, 114 aa, synthetic construct
  source 1..114: note = Light chain variable region of 4F1 germline reversion
DIVMTQSPLSLPVTPGEPASISCRSSQSLLHSNGYTYLDWYLQKPGQSPQLLIFLGSSRASGVPDRFSGSGSGTDFTLKISRVEAEDVGVYYCVQDLQTSLTFGGGTKLEIKRT

SEQ ID NO: 5 - protein, 114 aa, synthetic construct
  source 1..114: note = Light chain variable region of 4F1En3
DIVMTQSPLSLPVTPGEPASISCRSSQSLRHSNGYTYLDWYLQKPGQSPQLLIFLGSSRASGVPDRFSGSGSGTDFTLKISRVEAEDVGVYYCVQDLQTSLTFGGGTKLEIKRT

SEQ ID NO: 6 - protein, 114 aa, synthetic construct
  source 1..114: note = Light chain variable region of 4F1En4
DIVMTQSPLSLPVTPGEPASISCRSSQSLLHQNGYTYLDWYLQKPGQSPQLLIFLGSSRASGVPDRFSGSGSGTDFTLKISRVEAEDVGVYYCVQDLQTSLTFGGGTKLEIKRT

SEQ ID NO: 7 - protein, 114 aa, synthetic construct
  source 1..114: note = Light chain variable region of 4F1En5
DIVMTQSPLSLPVTPGEPASISCRSSQSLLHSNGYTYLDWYLQKPGQSPQLLIFLGSSRASGVPDRFSGSGQGTDFTLKISRVEAEDVGVYYCVQDLQTSLTFGGGTKLEIKRT

SEQ ID NO: 8 - DNA, 380 bp, synthetic construct
  source 1..380: mol_type = other DNA; note = Heavy chain variable region of 4F1 germline reversion
caggtgcagctcgtggagtctggcggcggcgtggtgcagccaggccggagcctcagactgtcttgcgctgccagcggcttcagcttctactcttactccgtgcactgggtgagacaggctccaggcaagggcttggagtgggtggctgacgtggtgtacgacggcaaccaccagcactacaccgactctgtgaagggcagattcacaattagcagggacacatccaagaacacagtgtacctacaaatgggctccctgagagccgaggacaccgccctgtactactgcaccgcccgatcgctcgtgatcaccctcgctggcgctggccgggacgactactggggccagggcacaacagtgaccgtgtcttccgcgtcgac

SEQ ID NO: 9 - DNA, 380 bp, synthetic construct
  source 1..380: mol_type = other DNA; note = Heavy chain variable region of 4F1En1
caggtgcagctcgtggagtctggcggcggcgtggtgcagccaggccggagcctcagactgtcttgcgctgccagcggcttcagcttctactcttactccgtgcactgggtgagacaggctccaggcaagggcttggagtgggtggctgacgtggtgtacgacggcaaccaccagcactacaccgactctgtgaagggcagattcacaattagcagggacacaagaaagaacacagtgtacctacaaatgggctccctgagagccgaggacaccgccctgtactactgcaccgcccgatcgctcgtgatcaccctcgctggcgctggccgggacgactactggggccagggcacaacagtgaccgtgtcttccgcgtcgac

SEQ ID NO: 10 - DNA, 380 bp, synthetic construct
  source 1..380: mol_type = other DNA; note = Heavy chain variable region of 4F1En2
caggtgcagctcgtggagtctggcggcggcgtggtgcagccaggccggagcctcagactgtcttgcgctgccagcggcttcagcttctactcttactccgtgcactgggtgagacaggctccaggcaagggcttggagtgggtggctgacgtggtgtacgacggcaaccaccagcactacaccgactctgtgaagggcagattcacaattagcagggacacaagaaagaacacagtgtacctacaaatgggctccctgagagccgaggacaccgccctgtactactgcaccgcccgatcgctcagcatcaccctcgctggcgctggccgggacgactactggggccagggcacaacagtgaccgtgtcttccgcgtcgac

SEQ ID NO: 11 - DNA, 342 bp, synthetic construct
  source 1..342: mol_type = other DNA; note = Light chain variable region of 4F1 germline reversion
gacatcgtgatgacccagtccccactgagcctccctgtgacaccaggcgagcccgcttctatctcttgccggtcttctcagagcctgctgcactctaacggctacacatacctcgactggtatctccagaagccaggccagtctccacagctgctcatcttcctcggcagctctagggccagcggcgtgcccgaccgcttctccggctctggctctggcaccgacttcacactcaagatcagcagagtggaggccgaggacgtgggcgtgtactactgcgtgcaggacctccagacatccctgacattcggcggcggcacaaagctggagatcaagcgtacg

SEQ ID NO: 12 - DNA, 342 bp, synthetic construct
  source 1..342: mol_type = other DNA; note = Light chain variable region of 4F1En3
gacatcgtgatgacccagtccccactgagcctccctgtgacaccaggcgagcccgcttctatctcttgccggtcttctcagagcctgaggcactctaacggctacacatacctcgactggtatctccagaagccaggccagtctccacagctgctcatcttcctcggcagctctagggccagcggcgtgcccgaccgcttctccggctctggctctggcaccgacttcacactcaagatcagcagagtggaggccgaggacgtgggcgtgtactactgcgtgcaggacctccagacatccctgacattcggcggcggcacaaagctggagatcaagcgtacg

SEQ ID NO: 13 - DNA, 342 bp, synthetic construct
  source 1..342: mol_type = other DNA; note = Light chain variable region of 4F1En4
gacatcgtgatgacccagtccccactgagcctccctgtgacaccaggcgagcccgcttctatctcttgccggtcttctcagagcctgctgcaccagaacggctacacatacctcgactggtatctccagaagccaggccagtctccacagctgctcatcttcctcggcagctctagggccagcggcgtgcccgaccgcttctccggctctggctctggcaccgacttcacactcaagatcagcagagtggaggccgaggacgtgggcgtgtactactgcgtgcaggacctccagacatccctgacattcggcggcggcacaaagctggagatcaagcgtacg

SEQ ID NO: 14 - DNA, 342 bp, synthetic construct
  source 1..342: mol_type = other DNA; note = Light chain variable region of 4F1En5
gacatcgtgatgacccagtccccactgagcctccctgtgacaccaggcgagcccgcttctatctcttgccggtcttctcagagcctgctgcactctaacggctacacatacctcgactggtatctccagaagccaggccagtctccacagctgctcatcttcctcggcagctctagggccagcggcgtgcccgaccgcttctccggctctggccagggcaccgacttcacactcaagatcagcagagtggaggccgaggacgtgggcgtgtactactgcgtgcaggacctccagacatccctgacattcggcggcggcacaaagctggagatcaagcgtacg

SEQ ID NO: 15 - protein, 124 aa, Homo sapiens
EVQLVQSGGGVVRPGRSLRLSCAASGFSFYSYSVHWVRQAPGKGLEWVADVVYDGNHQHYTESVRGRFSISRDTSTNTVYLQMGSLRPEDTALYYCTARSLVITLAGAGRDDYWGQGTRVTVSS

SEQ ID NO: 16 - protein, 112 aa, Homo sapiens
DIVMTQSPLSLSVTPGEPASISCKSSQSLLHSNGYTYLDWYLQKPGKSPQLLIFLGSSRASGVPARFSGSGSGTDFTLEISRVEAEDVGVYYCVQDLQTSLTFGGGTKVDIK

SEQ ID NO: 17 - DNA, 24 bp, synthetic construct
  source 1..24: mol_type = other DNA; note = RSV NP -sp
agatcaacttctgtcatccagcaa

SEQ ID NO: 18 - DNA, 29 bp, synthetic construct
  source 1..29: mol_type = other DNA; note = RSV NP -asp
ttctgcacatcataattaggagtatcaat

SEQ ID NO: 19 - DNA, 20 bp, synthetic construct
  source 1..20: mol_type = other DNA; note = mouse beta-actin-sp
ggctgtattcccctccatcg

SEQ ID NO: 20 - DNA, 22 bp, synthetic construct
  source 1..22: mol_type = other DNA; note = mouse beta-actin-asp
ccagttggtaacaatgccatgt